European Patent Specification EP 4 135 751 B1, published July 31, 2024. Title: IL-12 antagonists with optimized linkers. Applicant: Philogen S.p.A. The sequence listing filed with the application follows.

SEQUENCE LISTING (9 sequences)

SEQ ID NO: 1 - protein, 306 aa, Homo sapiens
IWELKKDVYVVELDWYPDAPGEMVVLTCDTPEEDGITWTLDQSSEVLGSGKTLTIQVKEFGDAGQYTCHKGGEVLSHSLLLLHKKEDGIWSTDILKDQKEPKNKTFLRCEAKNYSGRFTCWWLTTISTDLTFSVKSSRGSSDPQGVTCGAATLSAERVRGDNKEYEYSVECQEDSACPAAEESLPIEVMVDAVHKLKYENYTSSFFIRDIIKPDPPKNLQLKPLKNSRQVEVSWEYPDTWSTPHSYFSLTFCVQVQGKSKREKKDRVFTDKTSATVICRKNASISVRAQDRYYSSSWSEWASVPCS

SEQ ID NO: 2 - protein, 15 aa, artificial sequence
  linker
GGGGSGGGGSGGGGS

SEQ ID NO: 3 - protein, 197 aa, Homo sapiens
RNLPVATPDPGMFPCLHHSQNLLRAVSNMLQKARQTLEFYPCTSEEIDHEDITKDKTSTVEACLPLELTKNESCLNSRETSFITNGSCLASRKTSFMMALCLSSIYEDLKMYQVEFKTMNAKLLMDPKRQIFLDQNMLAVIDELMQALNFNSETVPQKSSLEEPDFYKTKIKLCILLHAFRIRAVTIDRVMSYLNAS

SEQ ID NO: 4 - protein, 15 aa, artificial sequence
  linker
GSADGGSSAGGSDAG

SEQ ID NO: 5 - protein, 108 aa, artificial sequence [sequence omitted]

SEQ ID NO: 6 - protein, 5 aa, artificial sequence
  linker
GSSGG

SEQ ID NO: 7 - protein, 116 aa, artificial sequence [sequence omitted]

SEQ ID NO: 8 - protein, 15 aa, artificial sequence
  linker
SSSSGSSSSGSSSSG

SEQ ID NO: 9 - protein, 1006 aa, artificial sequence
  Immunoconjugate sequence
IWELKKDVYVVELDWYPDAPGEMVVLTCDTPEEDGITWTLDQSSEVLGSGKTLTIQVKEFGDAGQYTCHKGGEVLSHSLLLLHKKEDGIWSTDILKDQKEPKNKTFLRCEAKNYSGRFTCWWLTTISTDLTFSVKSSRGSSDPQGVTCGAATLSAERVRGDNKEYEYSVECQEDSACPAAEESLPIEVMVDAVHKLKYENYTSSFFIRDIIKPDPPKNLQLKPLKNSRQVEVSWEYPDTWSTPHSYFSLTFCVQVQGKSKREKKDRVFTDKTSATVICRKNASISVRAQDRYYSSSWSEWASVPCSGGGGSGGGGSGGGGSRNLPVATPDPGMFPCLHHSQNLLRAVSNMLQKARQTLEFYPCTSEEIDHEDITKDKTSTVEACLPLELTKNESCLNSRETSFITNGSCLASRKTSFMMALCLSSIYEDLKMYQVEFKTMNAKLLMDPKRQIFLDQNMLAVIDELMQALNFNSETVPQKSSLEEPDFYKTKIKLCILLHAFRIRAVTIDRVMSYLNASGSADGGSSAGGSDAGEVQLLESGGGLVQPGGSLRLSCAASGFTFSSFSMSWVRQAPGKGLEWVSSISGSSGTTYYADSVKGRFTISRDNSKNTLYLQMNSLRAEDTAVYYCAKPFPYFDYWGQGTLVTVSSGSSGGEIVLTQSPGTLSLSPGERATLSCRASQSVSSSFLAWYQQKPGQAPRLLIYYASSRATGIPDRFSGSGSGTDFTLTISRLEPEDFAVYYCQQTGRIPPTFGQGTKVEIKSSSSGSSSSGSSSSGEVQLLESGGGLVQPGGSLRLSCAASGFTFSSFSMSWVRQAPGKGLEWVSSISGSSGTTYYADSVKGRFTISRDNSKNTLYLQMNSLRAEDTAVYYCAKPFPYFDYWGQGTLVTVSSGSSGGEIVLTQSPGTLSLSPGERATLSCRASQSVSSSFLAWYQQKPGQAPRLLIYYASSRATGIPDRFSGSGSGTDFTLTISRLEPEDFAVYYCQQTGRIPPTFGQGTKVEIK